European Patent Specification EP 3 702 471 B1, published December 24, 2025. Title: MODIFIED POLYMERASES FOR IMPROVED INCORPORATION OF NUCLEOTIDE ANALOGUES. Applicant: Illumina, Inc. The sequence listing filed with the application follows.

SEQUENCE LISTING (32 sequences)

SEQ ID NO: 1 - protein, 18 aa, Artificial Sequence
  Various including Thermococcus sp. or Pyrococcus sp.
  VARIANT (2)..(2): X= any AA
  VARIANT (3)..(3): X= any AA
  VARIANT (4)..(4): X= any AA
  VARIANT (8)..(8): X= any AA
  VARIANT (10)..(10): X= any AA
  VARIANT (11)..(11): X= any AA
  VARIANT (12)..(12): X= any AA
  VARIANT (14)..(14): X= any AA
EXXXLDYXQXXXKXLANS

SEQ ID NO: 2 - protein, 18 aa, Artificial Sequence
  Various including Thermococcus sp. or Pyrococcus sp.
  VARIANT (2)..(2): X=K, R, Y
  VARIANT (3)..(3): X=K, I, Q
  VARIANT (4)..(4): X=L, I, M
  VARIANT (8)..(8): X=R, E
  VARIANT (10)..(10): X=R, K, I
  VARIANT (11)..(11): X=A, K, L, V, S
  VARIANT (12)..(12): X=I, V, L, N
  VARIANT (14)..(14): X=I, V, L
EXXXLDYXQXXXKXLANS

SEQ ID NO: 3 - protein, 18 aa, Artificial Sequence
  Various including Thermococcus sp. or Pyrococcus sp.
  VARIANT (2)..(2): X=R, K
  VARIANT (3)..(3): X=K, I
  VARIANT (10)..(10): X=R, K
  VARIANT (14)..(14): X=I, L
EXXLLDYRQXAIKXLANS

SEQ ID NO: 4 - protein, 18 aa, Artificial Sequence
  Various including Thermococcus sp. or Pyrococcus sp.
EKKLLDYRQRAIKILANS

SEQ ID NO: 5 - protein, 775 aa, Thermococcus sp. 9N-7
MILDTDYITENGKPVIRVFKKENGEFKIEYDRTFEPYFYALLKDDSAIEDVKKVTAKRHGTVVKVKRAEKVQKKFLGRPIEVWKLYFNHPQDVPAIRDRIRAHPAVVDIYEYDIPFAKRYLIDKGLIPMEGDEELTMLAFDIETLYHEGEEFGTGPILMISYADGSEARVITWKKIDLPYVDVVSTEKEMIKRFLRVVREKDPDVLITYNGDNFDFAYLKKRCEELGIKFTLGRDGSEPKIQRMGDRFAVEVKGRIHFDLYPVIRRTINLPTYTLEAVYEAVFGKPKEKVYAEEIAQAWESGEGLERVARYSMEDAKVTYELGREFFPMEAQLSRLIGQSLWDVSRSSTGNLVEWFLLRKAYKRNELAPNKPDERELARRRGGYAGGYVKEPERGLWDNIVYLDFRSLYPSIIITHNVSPDTLNREGCKEYDVAPEVGHKFCKDFPGFIPSLLGDLLEERQKIKRKMKATVDPLEKKLLDYRQRAIKILANSFYGYYGYAKARWYCKECAESVTAWGREYIEMVIRELEEKFGFKVLYADTDGLHATIPGADAETVKKKAKEFLKYINPKLPGLLELEYEGFYVRGFFVTKKKYAVIDEEGKITTRGLEIVRRDWSEIAKETQARVLEAILKHGDVEEAVRIVKEVTEKLSKYEVPPEKLVIHEQITRDLRDYKATGPHVAVAKRLAARGVKIRPGTVISYIVLKGSGRIGDRAIPADEFDPTKHRYDAEYYIENQVLPAVERILKAFGYRKEDLRYQKTKQVGLGAWLKVKGKK

SEQ ID NO: 6 - protein, 775 aa, Thermococcus sp. 9N-7
MILDTDYITENGKPVIRVFKKENGEFKIEYDRTFEPYFYALLKDDSAIEDVKKVTAKRHGTVVKVKRAEKVQKKFLGRPIEVWKLYFNHPQDVPAIRDRIRAHPAVVDIYEYDIPFAKRYLIDKGLIPMEGDEELTMLAFDIETLYHEGEEFGTGPILMISYADGSEARVITWKKIDLPYVDVVSTEKEMIKRFLRVVREKDPDVLITYNGDNFDFAYLKKRCEELGIKFTLGRDGSEPKIQRMGDRFAVEVKGRIHFDLYPVIRRTINLPTYTLEAVYEAVFGKPKEKVYAEEIAQAWESGEGLERVARYSMEDAKVTYELGREFFPMEAQLSRLIGQSLWDVSRSSTGNLVEWFLLRKAYKRNELAPNKPDERELARRRGGYAGGYVKEPERGLWDNIVYLDFRSLYPSIIITHNVSPDTLNREGCKEYDVAPEVGHKFCKDFPGFIPSLLGDLLEERQKIKRKMKATVDPLEKMLLDYRQRAIKILANSFYGYYGYAKARWYCKECAESVTAWGREYIEMVIRELEEKFGFKVLYADTDGLHATIPGADAETVKKKAKEFLKYINPKLPGLLELEYEGFYVRGFFVTKKKYAVIDEEGKITTRGLEIVRRDWSEIAKETQARVLEAILKHGDVEEAVRIVKEVTEKLSKYEVPPEKLVIHEQITRDLRDYKATGPHVAVAKRLAARGVKIRPGTVISYIVLKGSGRIGDRAIPADEFDPTKHRYDAEYYIENQVLPAVERILKAFGYRKEDLRYQKTKQVGLGAWLKVKGKK

SEQ ID NO: 7 - protein, 775 aa, Thermococcus sp. 9N-7
  VARIANT (410)..(410): X=I, V, A
MILDTDYITENGKPVIRVFKKENGEFKIEYDRTFEPYFYALLKDDSAIEDVKKVTAKRHGTVVKVKRAEKVQKKFLGRPIEVWKLYFNHPQDVPAIRDRIRAHPAVVDIYEYDIPFAKRYLIDKGLIPMEGDEELTMLAFDIETLYHEGEEFGTGPILMISYADGSEARVITWKKIDLPYVDVVSTEKEMIKRFLRVVREKDPDVLITYNGDNFDFAYLKKRCEELGIKFTLGRDGSEPKIQRMGDRFAVEVKGRIHFDLYPVIRRTINLPTYTLEAVYEAVFGKPKEKVYAEEIAQAWESGEGLERVARYSMEDAKVTYELGREFFPMEAQLSRLIGQSLWDVSRSSTGNLVEWFLLRKAYKRNELAPNKPDERELARRRGGYAGGYVKEPERGLWDNIVYLDFRSAAXSIIITHNVSPDTLNREGCKEYDVAPEVGHKFCKDFPGFIPSLLGDLLEERQKIKRKMKATVDPLEKMLLDYRQRAIKILANSFYGYYGYAKARWYCKECAESVTAWGREYIEMVIRELEEKFGFKVLYADTDGLHATIPGADAETVKKKAKEFLKYINPKLPGLLELEYEGFYVRGFFVTKKKYAVIDEEGKITTRGLEIVRRDWSEIAKETQARVLEAILKHGDVEEAVRIVKEVTEKLSKYEVPPEKLVIHEQITRDLRDYKATGPHVAVAKRLAARGVKIRPGTVISYIVLKGSGRIGDRAIPADEFDPTKHRYDAEYYIENQVLPAVERILKAFGYRKEDLRYQKTKQVGLGAWLKVKGKK

SEQ ID NO: 8 - protein, 775 aa, Thermococcus sp. 9N-7
MILDTDYITENGKPVIRVFKKENGEFKIEYDRTFEPYFYALLKDDSAIEDVKKVTAKRHGTVVKVKRAEKVQKKFLGRPIEVWKLYFNHPQDVPAIRDRIRAHPAVVDIYEYDIPFAKRYLIDKGLIPMEGDEELTMLAFDIETLYHEGEEFGTGPILMISYADGSEARVITWKKIDLPYVDVVSTEKEMIKRFLRVVREKDPDVLITYNGDNFDFAYLKKRCEELGIKFTLGRDGSEPKIQRMGDRFAVEVKGRIHFDLYPVIRRTINLPTYTLEAVYEAVFGKPKEKVYAEEIAQAWESGEGLERVARYSMEDAKVTYELGREFFPMEAQLSRLIGQSLWDVSRSSTGNLVEWFLLRKAYKRNELAPNKPDERELARRRGGYAGGYVKEPERGLWDNIVYLDFRSLAPSIIITHNVSPDTLNREGCKEYDVAPEVGHKFCKDFPGFIPSLLGDLLEERQKIKRKMKATVDPLEKMLLDYRQRAIKILANSFYGYYGYAKARWYCKECAESVTAWGREYIEMVIRELEEKFGFKVLYADTDGLHATIPGADAETVKKKAKEFLKYINPKLPGLLELEYEGFYVRGFFVTKKKYAVIDEEGKITTRGLEIVRRDWSEIAKETQARVLEAILKHGDVEEAVRIVKEVTEKLSKYEVPPEKLVIHEQITRDLRDYKATGPHVAVAKRLAARGVKIRPGTVISYIVLKGSGRIGDRAIPADEFDPTKHRYDAEYYIENQVLPAVERILKAFGYRKEDLRYQKTKQVGLGAWLKVKGKK

SEQ ID NO: 9 - protein, 775 aa, Thermococcus sp. 9N-7
MILDTDYITENGKPVIRVFKKENGEFKIEYDRTFEPYFYALLKDDSAIEDVKKVTAKRHGTVVKVKRAEKVQKKFLGRPIEVWKLYFNHPQDVPAIRDRIRAHPAVVDIYEYDIPFAKRYLIDKGLIPMEGDEELTMLAFAIATLYHEGEEFGTGPILMISYADGSEARVITWKKIDLPYVDVVSTEKEMIKRFLRVVREKDPDVLITYNGDNFDFAYLKKRCEELGIKFTLGRDGSEPKIQRMGDRFAVEVKGRIHFDLYPVIRRTINLPTYTLEAVYEAVFGKPKEKVYAEEIAQAWESGEGLERVARYSMEDAKVTYELGREFFPMEAQLSRLIGQSLWDVSRSSTGNLVEWFLLRKAYKRNELAPNKPDERELARRRGGYAGGYVKEPERGLWDNIVYLDFRSLYPSIIITHNVSPDTLNREGCKEYDVAPEVGHKFCKDFPGFIPSLLGDLLEERQKIKRKMKATVDPLEKKLLDYRQRAIKILANSFYGYYGYAKARWYCKECAESVTAWGREYIEMVIRELEEKFGFKVLYADTDGLHATIPGADAETVKKKAKEFLKYINPKLPGLLELEYEGFYVRGFFVTKKKYAVIDEEGKITTRGLEIVRRDWSEIAKETQARVLEAILKHGDVEEAVRIVKEVTEKLSKYEVPPEKLVIHEQITRDLRDYKATGPHVAVAKRLAARGVKIRPGTVISYIVLKGSGRIGDRAIPADEFDPTKHRYDAEYYIENQVLPAVERILKAFGYRKEDLRYQKTKQVGLGAWLKVKGKK

SEQ ID NO: 10 - protein, 775 aa, Thermococcus sp. 9N-7
MILDTDYITENGKPVIRVFKKENGEFKIEYDRTFEPYFYALLKDDSAIEDVKKVTAKRHGTVVKVKRAEKVQKKFLGRPIEVWKLYFNHPQDVPAIRDRIRAHPAVVDIYEYDIPFAKRYLIDKGLIPMEGDEELTMLAFAIATLYHEGEEFGTGPILMISYADGSEARVITWKKIDLPYVDVVSTEKEMIKRFLRVVREKDPDVLITYNGDNFDFAYLKKRCEELGIKFTLGRDGSEPKIQRMGDRFAVEVKGRIHFDLYPVIRRTINLPTYTLEAVYEAVFGKPKEKVYAEEIAQAWESGEGLERVARYSMEDAKVTYELGREFFPMEAQLSRLIGQSLWDVSRSSTGNLVEWFLLRKAYKRNELAPNKPDERELARRRGGYAGGYVKEPERGLWDNIVYLDFRSLYPSIIITHNVSPDTLNREGCKEYDVAPEVGHKFCKDFPGFIPSLLGDLLEERQKIKRKMKATVDPLEKMLLDYRQRAIKILANSFYGYYGYAKARWYCKECAESVTAWGREYIEMVIRELEEKFGFKVLYADTDGLHATIPGADAETVKKKAKEFLKYINPKLPGLLELEYEGFYVRGFFVTKKKYAVIDEEGKITTRGLEIVRRDWSEIAKETQARVLEAILKHGDVEEAVRIVKEVTEKLSKYEVPPEKLVIHEQITRDLRDYKATGPHVAVAKRLAARGVKIRPGTVISYIVLKGSGRIGDRAIPADEFDPTKHRYDAEYYIENQVLPAVERILKAFGYRKEDLRYQKTKQVGLGAWLKVKGKK

SEQ ID NO: 11 - protein, 775 aa, Thermococcus sp. 9N-7
  VARIANT (410)..(410): X=I, V, A
MILDTDYITENGKPVIRVFKKENGEFKIEYDRTFEPYFYALLKDDSAIEDVKKVTAKRHGTVVKVKRAEKVQKKFLGRPIEVWKLYFNHPQDVPAIRDRIRAHPAVVDIYEYDIPFAKRYLIDKGLIPMEGDEELTMLAFAIATLYHEGEEFGTGPILMISYADGSEARVITWKKIDLPYVDVVSTEKEMIKRFLRVVREKDPDVLITYNGDNFDFAYLKKRCEELGIKFTLGRDGSEPKIQRMGDRFAVEVKGRIHFDLYPVIRRTINLPTYTLEAVYEAVFGKPKEKVYAEEIAQAWESGEGLERVARYSMEDAKVTYELGREFFPMEAQLSRLIGQSLWDVSRSSTGNLVEWFLLRKAYKRNELAPNKPDERELARRRGGYAGGYVKEPERGLWDNIVYLDFRSAAXSIIITHNVSPDTLNREGCKEYDVAPEVGHKFCKDFPGFIPSLLGDLLEERQKIKRKMKATVDPLEKMLLDYRQRAIKILANSFYGYYGYAKARWYCKECAESVTAWGREYIEMVIRELEEKFGFKVLYADTDGLHATIPGADAETVKKKAKEFLKYINPKLPGLLELEYEGFYVRGFFVTKKKYAVIDEEGKITTRGLEIVRRDWSEIAKETQARVLEAILKHGDVEEAVRIVKEVTEKLSKYEVPPEKLVIHEQITRDLRDYKATGPHVAVAKRLAARGVKIRPGTVISYIVLKGSGRIGDRAIPADEFDPTKHRYDAEYYIENQVLPAVERILKAFGYRKEDLRYQKTKQVGLGAWLKVKGKK

SEQ ID NO: 12 - protein, 775 aa, Thermococcus sp. 9N-7
MILDTDYITENGKPVIRVFKKENGEFKIEYDRTFEPYFYALLKDDSAIEDVKKVTAKRHGTVVKVKRAEKVQKKFLGRPIEVWKLYFNHPQDVPAIRDRIRAHPAVVDIYEYDIPFAKRYLIDKGLIPMEGDEELTMLAFAIATLYHEGEEFGTGPILMISYADGSEARVITWKKIDLPYVDVVSTEKEMIKRFLRVVREKDPDVLITYNGDNFDFAYLKKRCEELGIKFTLGRDGSEPKIQRMGDRFAVEVKGRIHFDLYPVIRRTINLPTYTLEAVYEAVFGKPKEKVYAEEIAQAWESGEGLERVARYSMEDAKVTYELGREFFPMEAQLSRLIGQSLWDVSRSSTGNLVEWFLLRKAYKRNELAPNKPDERELARRRGGYAGGYVKEPERGLWDNIVYLDFRSLAPSIIITHNVSPDTLNREGCKEYDVAPEVGHKFCKDFPGFIPSLLGDLLEERQKIKRKMKATVDPLEKMLLDYRQRAIKILANSFYGYYGYAKARWYCKECAESVTAWGREYIEMVIRELEEKFGFKVLYADTDGLHATIPGADAETVKKKAKEFLKYINPKLPGLLELEYEGFYVRGFFVTKKKYAVIDEEGKITTRGLEIVRRDWSEIAKETQARVLEAILKHGDVEEAVRIVKEVTEKLSKYEVPPEKLVIHEQITRDLRDYKATGPHVAVAKRLAARGVKIRPGTVISYIVLKGSGRIGDRAIPADEFDPTKHRYDAEYYIENQVLPAVERILKAFGYRKEDLRYQKTKQVGLGAWLKVKGKK

SEQ ID NO: 13 - protein, 775 aa, Thermococcus sp. 9N-7
MILDTDYITENGKPVIRVFKKENGEFKIEYDRTFEPYFYALLKDDSAIEDVKKVTAKRHGTVVKVKRAEKVQKKFLGRPIEVWKLYFNHPQDVPAIRDRIRAHPAVVDIYEYDIPFAKRYLIDKGLIPMEGDEELTMLAFAIATLYHEGEEFGTGPILMISYADGSEARVITWKKIDLPYVDVVSTEKEMIKRFLRVVREKDPDVLITYNGDNFDFAYLKKRSEELGIKFTLGRDGSEPKIQRMGDRFAVEVKGRIHFDLYPVIRRTINLPTYTLEAVYEAVFGKPKEKVYAEEIAQAWESGEGLERVARYSMEDAKVTYELGREFFPMEAQLSRLIGQSLWDVSRSSTGNLVEWFLLRKAYKRNELAPNKPDERELARRRGGYAGGYVKEPERGLWDNIVYLDFRSAAASIIITHNVSPDTLNREGCKEYDVAPEVGHKFCKDFPGFIPSLLGDLLEERQKIKRKMKATVDPLEKKLLDYRQRLIKILANSFYGYYGYAKARWYCKECAESVTAWGREYIEMVIRELEEKFGFKVLYADTDGLHATIPGADAETVKKKAKEFLKYINPKLPGLLELEYEGFYVRGFFVTKKKYAVIDEEGKITTRGLEIVRRDWSEIAKETQARVLEAILKHGDVEEAVRIVKEVTEKLSKYEVPPEKLVIHEQITRDLRDYKATGPHVAVAKRLAARGVKIRPGTVISYIVLKGSGRIGDRAIPADEFDPTKHRYDAEYYIENQVLPAVERILKAFGYRKEDLRYQKTKQVGLGAWLKVKGKK

SEQ ID NO: 14 - protein, 775 aa, Thermococcus sp. 9N-7
MILDTDYITENGKPVIRVFKKENGEFKIEYDRTFEPYFYALLKDDSAIEDVKKVTAKRHGTVVKVKRAEKVQKKFLGRPIEVWKLYFNHPQDVPAIRDRIRAHPAVVDIYEYDIPFAKRYLIDKGLIPMEGDEELTMLAFAIATLYHEGEEFGTGPILMISYADGSEARVITWKKIDLPYVDVVSTEKEMIKRFLRVVREKDPDVLITYNGDNFDFAYLKKRSEELGIKFTLGRDGSEPKIQRMGDRFAVEVKGRIHFDLYPVIRRTINLPTYTLEAVYEAVFGKPKEKVYAEEIAQAWESGEGLERVARYSMEDAKVTYELGREFFPMEAQLSRLIGQSLWDVSRSSTGNLVEWFLLRKAYKRNELAPNKPDERELARRRGGYAGGYVKEPERGLWDNIVYLDFRSAAASIIITHNVSPDTLNREGCKEYDVAPEVGHKFCKDFPGFIPSLLGDLLEERQKIKRKMKATVDPLEKMLLDYRQRLIKILANSFYGYYGYAKARWYCKECAESVTAWGREYIEMVIRELEEKFGFKVLYADTDGLHATIPGADAETVKKKAKEFLKYINPKLPGLLELEYEGFYVRGFFVTKKKYAVIDEEGKITTRGLEIVRRDWSEIAKETQARVLEAILKHGDVEEAVRIVKEVTEKLSKYEVPPEKLVIHEQITRDLRDYKATGPHVAVAKRLAARGVKIRPGTVISYIVLKGSGRIGDRAIPADEFDPTKHRYDAEYYIENQVLPAVERILKAFGYRKEDLRYQKTKQVGLGAWLKVKGKK

SEQ ID NO: 15 - protein, 775 aa, Thermococcus sp. 9N-7
  VARIANT (410)..(410): X=I, V, A
MILDTDYITENGKPVIRVFKKENGEFKIEYDRTFEPYFYALLKDDSAIEDVKKVTAKRHGTVVKVKRAEKVQKKFLGRPIEVWKLYFNHPQDVPAIRDRIRAHPAVVDIYEYDIPFAKRYLIDKGLIPMEGDEELTMLAFAIATLYHEGEEFGTGPILMISYADGSEARVITWKKIDLPYVDVVSTEKEMIKRFLRVVREKDPDVLITYNGDNFDFAYLKKRSEELGIKFTLGRDGSEPKIQRMGDRFAVEVKGRIHFDLYPVIRRTINLPTYTLEAVYEAVFGKPKEKVYAEEIAQAWESGEGLERVARYSMEDAKVTYELGREFFPMEAQLSRLIGQSLWDVSRSSTGNLVEWFLLRKAYKRNELAPNKPDERELARRRGGYAGGYVKEPERGLWDNIVYLDFRSAAXSIIITHNVSPDTLNREGCKEYDVAPEVGHKFCKDFPGFIPSLLGDLLEERQKIKRKMKATVDPLEKMLLDYRQRLIKILANSFYGYYGYAKARWYCKECAESVTAWGREYIEMVIRELEEKFGFKVLYADTDGLHATIPGADAETVKKKAKEFLKYINPKLPGLLELEYEGFYVRGFFVTKKKYAVIDEEGKITTRGLEIVRRDWSEIAKETQARVLEAILKHGDVEEAVRIVKEVTEKLSKYEVPPEKLVIHEQITRDLRDYKATGPHVAVAKRLAARGVKIRPGTVISYIVLKGSGRIGDRAIPADEFDPTKHRYDAEYYIENQVLPAVERILKAFGYRKEDLRYQKTKQVGLGAWLKVKGKK

SEQ ID NO: 16 - protein, 775 aa, Thermococcus sp. 9N-7
MILDTDYITENGKPVIRVFKKENGEFKIEYDRTFEPYFYALLKDDSAIEDVKKVTAKRHGTVVKVKRAEKVQKKFLGRPIEVWKLYFNHPQDVPAIRDRIRAHPAVVDIYEYDIPFAKRYLIDKGLIPMEGDEELTMLAFAIATLYHEGEEFGTGPILMISYADGSEARVITWKKIDLPYVDVVSTEKEMIKRFLRVVREKDPDVLITYNGDNFDFAYLKKRSEELGIKFTLGRDGSEPKIQRMGDRFAVEVKGRIHFDLYPVIRRTINLPTYTLEAVYEAVFGKPKEKVYAEEIAQAWESGEGLERVARYSMEDAKVTYELGREFFPMEAQLSRLIGQSLWDVSRSSTGNLVEWFLLRKAYKRNELAPNKPDERELARRRGGYAGGYVKEPERGLWDNIVYLDFRSLAPSIIITHNVSPDTLNREGCKEYDVAPEVGHKFCKDFPGFIPSLLGDLLEERQKIKRKMKATVDPLEKMLLDYRQRLIKILANSFYGYYGYAKARWYCKECAESVTAWGREYIEMVIRELEEKFGFKVLYADTDGLHATIPGADAETVKKKAKEFLKYINPKLPGLLELEYEGFYVRGFFVTKKKYAVIDEEGKITTRGLEIVRRDWSEIAKETQARVLEAILKHGDVEEAVRIVKEVTEKLSKYEVPPEKLVIHEQITRDLRDYKATGPHVAVAKRLAARGVKIRPGTVISYIVLKGSGRIGDRAIPADEFDPTKHRYDAEYYIENQVLPAVERILKAFGYRKEDLRYQKTKQVGLGAWLKVKGKK

SEQ ID NO: 17 - protein, 775 aa, Pyrococcus furiosus
MILDVDYITEEGKPVIRLFKKENGKFKIEHDRTFRPYIYALLRDDSKIEEVKKITGERHGKIVRIVDVEKVEKKFLGKPITVWKLYLEHPQDVPTIREKVREHPAVVDIFEYDIPFAKRYLIDKGLIPMEGEEELKILAFAIATLYHEGEEFGKGPIIMISYADENEAKVITWKNIDLPYVEVVSSEREMIKRFLRIIREKDPDIIVTYNGDSFDFPYLAKRAEKLGIKLTIGRDGSEPKMQRIGDMTAVEVKGRIHFDLYHVITRTINLPTYTLEAVYEAIFGKPKEKVYADEIAKAWESGENLERVAKYSMEDAKATYELGKEFLPMEIQLSRLVGQPLWDVSRSSTGNLVEWFLLRKAYERNEVAPNKPSEEEYQRRLRESYTGGFVKEPEKGLWENIVYLDFRALYPSIIITHNVSPDTLNLEGCKNYDIAPQVGHKFCKDIPGFIPSLLGHLLEERQKIKTKMKETQDPIEKILLDYRQKLIKLLANSFYGYYGYAKARWYCKECAESVTAWGRKYIELVWKELEEKFGFKVLYIDTDGLYATIPGGESEEIKKKALEFVKYINSKLPGLLELEYEGFYKRGFFVTKKRYAVIDEEGKVITRGLEIVRRDWSEIAKETQARVLETILKHGDVEEAVRIVKEVIQKLANYEIPPEKLAIYEQITRPLHEYKAIGPHVAVAKKLAAKGVKIKPGMVIGYIVLRGDGPISNRAILAEEYDPKKHKYDAEYYIENQVLPAVLRILEGFGYRKEDLRYQKTRQVGLTSWLNIKKS

SEQ ID NO: 18 - protein, 775 aa, Pyrococcus furiosus
MILDVDYITEEGKPVIRLFKKENGKFKIEHDRTFRPYIYALLRDDSKIEEVKKITGERHGKIVRIVDVEKVEKKFLGKPITVWKLYLEHPQDVPTIREKVREHPAVVDIFEYDIPFAKRYLIDKGLIPMEGEEELKILAFAIATLYHEGEEFGKGPIIMISYADENEAKVITWKNIDLPYVEVVSSEREMIKRFLRIIREKDPDIIVTYNGDSFDFPYLAKRAEKLGIKLTIGRDGSEPKMQRIGDMTAVEVKGRIHFDLYHVITRTINLPTYTLEAVYEAIFGKPKEKVYADEIAKAWESGENLERVAKYSMEDAKATYELGKEFLPMEIQLSRLVGQPLWDVSRSSTGNLVEWFLLRKAYERNEVAPNKPSEEEYQRRLRESYTGGFVKEPEKGLWENIVYLDFRALYPSIIITHNVSPDTLNLEGCKNYDIAPQVGHKFCKDIPGFIPSLLGHLLEERQKIKTKMKETQDPIEKMLLDYRQKLIKLLANSFYGYYGYAKARWYCKECAESVTAWGRKYIELVWKELEEKFGFKVLYIDTDGLYATIPGGESEEIKKKALEFVKYINSKLPGLLELEYEGFYKRGFFVTKKRYAVIDEEGKVITRGLEIVRRDWSEIAKETQARVLETILKHGDVEEAVRIVKEVIQKLANYEIPPEKLAIYEQITRPLHEYKAIGPHVAVAKKLAAKGVKIKPGMVIGYIVLRGDGPISNRAILAEEYDPKKHKYDAEYYIENQVLPAVLRILEGFGYRKEDLRYQKTRQVGLTSWLNIKKS

SEQ ID NO: 19 - protein, 775 aa, Pyrococcus furiosus
  VARIANT (411)..(411): X=I, V, A
MILDVDYITEEGKPVIRLFKKENGKFKIEHDRTFRPYIYALLRDDSKIEEVKKITGERHGKIVRIVDVEKVEKKFLGKPITVWKLYLEHPQDVPTIREKVREHPAVVDIFEYDIPFAKRYLIDKGLIPMEGEEELKILAFAIATLYHEGEEFGKGPIIMISYADENEAKVITWKNIDLPYVEVVSSEREMIKRFLRIIREKDPDIIVTYNGDSFDFPYLAKRAEKLGIKLTIGRDGSEPKMQRIGDMTAVEVKGRIHFDLYHVITRTINLPTYTLEAVYEAIFGKPKEKVYADEIAKAWESGENLERVAKYSMEDAKATYELGKEFLPMEIQLSRLVGQPLWDVSRSSTGNLVEWFLLRKAYERNEVAPNKPSEEEYQRRLRESYTGGFVKEPEKGLWENIVYLDFRAAAXSIIITHNVSPDTLNLEGCKNYDIAPQVGHKFCKDIPGFIPSLLGHLLEERQKIKTKMKETQDPIEKMLLDYRQKLIKLLANSFYGYYGYAKARWYCKECAESVTAWGRKYIELVWKELEEKFGFKVLYIDTDGLYATIPGGESEEIKKKALEFVKYINSKLPGLLELEYEGFYKRGFFVTKKRYAVIDEEGKVITRGLEIVRRDWSEIAKETQARVLETILKHGDVEEAVRIVKEVIQKLANYEIPPEKLAIYEQITRPLHEYKAIGPHVAVAKKLAAKGVKIKPGMVIGYIVLRGDGPISNRAILAEEYDPKKHKYDAEYYIENQVLPAVLRILEGFGYRKEDLRYQKTRQVGLTSWLNIKKS

SEQ ID NO: 20 - protein, 775 aa, Pyrococcus furiosus
MILDVDYITEEGKPVIRLFKKENGKFKIEHDRTFRPYIYALLRDDSKIEEVKKITGERHGKIVRIVDVEKVEKKFLGKPITVWKLYLEHPQDVPTIREKVREHPAVVDIFEYDIPFAKRYLIDKGLIPMEGEEELKILAFAIATLYHEGEEFGKGPIIMISYADENEAKVITWKNIDLPYVEVVSSEREMIKRFLRIIREKDPDIIVTYNGDSFDFPYLAKRAEKLGIKLTIGRDGSEPKMQRIGDMTAVEVKGRIHFDLYHVITRTINLPTYTLEAVYEAIFGKPKEKVYADEIAKAWESGENLERVAKYSMEDAKATYELGKEFLPMEIQLSRLVGQPLWDVSRSSTGNLVEWFLLRKAYERNEVAPNKPSEEEYQRRLRESYTGGFVKEPEKGLWENIVYLDFRALAPSIIITHNVSPDTLNLEGCKNYDIAPQVGHKFCKDIPGFIPSLLGHLLEERQKIKTKMKETQDPIEKMLLDYRQKLIKLLANSFYGYYGYAKARWYCKECAESVTAWGRKYIELVWKELEEKFGFKVLYIDTDGLYATIPGGESEEIKKKALEFVKYINSKLPGLLELEYEGFYKRGFFVTKKRYAVIDEEGKVITRGLEIVRRDWSEIAKETQARVLETILKHGDVEEAVRIVKEVIQKLANYEIPPEKLAIYEQITRPLHEYKAIGPHVAVAKKLAAKGVKIKPGMVIGYIVLRGDGPISNRAILAEEYDPKKHKYDAEYYIENQVLPAVLRILEGFGYRKEDLRYQKTRQVGLTSWLNIKKS

SEQ ID NO: 21 - protein, 774 aa, Thermococcus kodakaraensis
MILDTDYITEDGKPVIRIFKKENGEFKIEYDRTFEPYFYALLKDDSAIEEVKKITAERHGTVVTVKRVEKVQKKFLGRPVEVWKLYFTHPQDVPAIRDKIREHPAVIDIYEYDIPFAKRYLIDKGLVPMEGDEELKMLAFAIATLYHEGEEFAEGPILMISYADEEGARVITWKNVDLPYVDVVSTEREMIKRFLRVVKEKDPDVLITYNGDNFDFAYLKKRCEKLGINFALGRDGSEPKIQRMGDRFAVEVKGRIHFDLYPVIRRTINLPTYTLEAVYEAVFGQPKEKVYAEEITTAWETGENLERVARYSMEDAKVTYELGKEFLPMEAQLSRLIGQSLWDVSRSSTGNLVEWFLLRKAYERNELAPNKPDEKELARRRQSYEGGYVKEPERGLWENIVYLDFRSLYPSIIITHNVSPDTLNREGCKEYDVAPQVGHRFCKDFPGFIPSLLGDLLEERQKIKKKMKATIDPIERKLLDYRQRLIKILANSYYGYYGYARARWYCKECAESVTAWGREYITMTIKEIEEKYGFKVIYSDTDGFFATIPGADAETVKKKAMEFLKYINAKLPGALELEYEGFYKRGFFVTKKKYAVIDEEGKITTRGLEIVRRDWSEIAKETQARVLEALLKDGDVEKAVRIVKEVTEKLSKYEVPPEKLVIHEQITRDLKDYKATGPHVAVAKRLAARGVKIRPGTVISYIVLKGSGRIGDRAIPFDEFDPTKHKYDAEYYIENQVLPAVERILRAFGYRKEDLRYQKTRQVGLSAWLKPKGT

SEQ ID NO: 22 - protein, 774 aa, Thermococcus kodakaraensis
MILDTDYITEDGKPVIRIFKKENGEFKIEYDRTFEPYFYALLKDDSAIEEVKKITAERHGTVVTVKRVEKVQKKFLGRPVEVWKLYFTHPQDVPAIRDKIREHPAVIDIYEYDIPFAKRYLIDKGLVPMEGDEELKMLAFAIATLYHEGEEFAEGPILMISYADEEGARVITWKNVDLPYVDVVSTEREMIKRFLRVVKEKDPDVLITYNGDNFDFAYLKKRCEKLGINFALGRDGSEPKIQRMGDRFAVEVKGRIHFDLYPVIRRTINLPTYTLEAVYEAVFGQPKEKVYAEEITTAWETGENLERVARYSMEDAKVTYELGKEFLPMEAQLSRLIGQSLWDVSRSSTGNLVEWFLLRKAYERNELAPNKPDEKELARRRQSYEGGYVKEPERGLWENIVYLDFRSLYPSIIITHNVSPDTLNREGCKEYDVAPQVGHRFCKDFPGFIPSLLGDLLEERQKIKKKMKATIDPIERMLLDYRQRLIKILANSYYGYYGYARARWYCKECAESVTAWGREYITMTIKEIEEKYGFKVIYSDTDGFFATIPGADAETVKKKAMEFLKYINAKLPGALELEYEGFYKRGFFVTKKKYAVIDEEGKITTRGLEIVRRDWSEIAKETQARVLEALLKDGDVEKAVRIVKEVTEKLSKYEVPPEKLVIHEQITRDLKDYKATGPHVAVAKRLAARGVKIRPGTVISYIVLKGSGRIGDRAIPFDEFDPTKHKYDAEYYIENQVLPAVERILRAFGYRKEDLRYQKTRQVGLSAWLKPKGT

SEQ ID NO: 23 - protein, 774 aa, Thermococcus kodakaraensis
  VARIANT (410)..(410): x=I, V, A
MILDTDYITEDGKPVIRIFKKENGEFKIEYDRTFEPYFYALLKDDSAIEEVKKITAERHGTVVTVKRVEKVQKKFLGRPVEVWKLYFTHPQDVPAIRDKIREHPAVIDIYEYDIPFAKRYLIDKGLVPMEGDEELKMLAFAIATLYHEGEEFAEGPILMISYADEEGARVITWKNVDLPYVDVVSTEREMIKRFLRVVKEKDPDVLITYNGDNFDFAYLKKRCEKLGINFALGRDGSEPKIQRMGDRFAVEVKGRIHFDLYPVIRRTINLPTYTLEAVYEAVFGQPKEKVYAEEITTAWETGENLERVARYSMEDAKVTYELGKEFLPMEAQLSRLIGQSLWDVSRSSTGNLVEWFLLRKAYERNELAPNKPDEKELARRRQSYEGGYVKEPERGLWENIVYLDFRSAAXSIIITHNVSPDTLNREGCKEYDVAPQVGHRFCKDFPGFIPSLLGDLLEERQKIKKKMKATIDPIERMLLDYRQRLIKILANSYYGYYGYARARWYCKECAESVTAWGREYITMTIKEIEEKYGFKVIYSDTDGFFATIPGADAETVKKKAMEFLKYINAKLPGALELEYEGFYKRGFFVTKKKYAVIDEEGKITTRGLEIVRRDWSEIAKETQARVLEALLKDGDVEKAVRIVKEVTEKLSKYEVPPEKLVIHEQITRDLKDYKATGPHVAVAKRLAARGVKIRPGTVISYIVLKGSGRIGDRAIPFDEFDPTKHKYDAEYYIENQVLPAVERILRAFGYRKEDLRYQKTRQVGLSAWLKPKGT

SEQ ID NO: 24 - protein, 774 aa, Thermococcus kodakaraensis
MILDTDYITEDGKPVIRIFKKENGEFKIEYDRTFEPYFYALLKDDSAIEEVKKITAERHGTVVTVKRVEKVQKKFLGRPVEVWKLYFTHPQDVPAIRDKIREHPAVIDIYEYDIPFAKRYLIDKGLVPMEGDEELKMLAFAIATLYHEGEEFAEGPILMISYADEEGARVITWKNVDLPYVDVVSTEREMIKRFLRVVKEKDPDVLITYNGDNFDFAYLKKRCEKLGINFALGRDGSEPKIQRMGDRFAVEVKGRIHFDLYPVIRRTINLPTYTLEAVYEAVFGQPKEKVYAEEITTAWETGENLERVARYSMEDAKVTYELGKEFLPMEAQLSRLIGQSLWDVSRSSTGNLVEWFLLRKAYERNELAPNKPDEKELARRRQSYEGGYVKEPERGLWENIVYLDFRSLAPSIIITHNVSPDTLNREGCKEYDVAPQVGHRFCKDFPGFIPSLLGDLLEERQKIKKKMKATIDPIERMLLDYRQRLIKILANSYYGYYGYARARWYCKECAESVTAWGREYITMTIKEIEEKYGFKVIYSDTDGFFATIPGADAETVKKKAMEFLKYINAKLPGALELEYEGFYKRGFFVTKKKYAVIDEEGKITTRGLEIVRRDWSEIAKETQARVLEALLKDGDVEKAVRIVKEVTEKLSKYEVPPEKLVIHEQITRDLKDYKATGPHVAVAKRLAARGVKIRPGTVISYIVLKGSGRIGDRAIPFDEFDPTKHKYDAEYYIENQVLPAVERILRAFGYRKEDLRYQKTRQVGLSAWLKPKGT

SEQ ID NO: 25 - protein, 784 aa, Methanococcus maripaludis
MESLIDLDYNSDDLCIYLYLINSIIKEKDFKPYFYVNSTDKEQILEFLKDYEKKHKLDSEISKMIENIETVKKIVFDENYQEKELSKVTVKYPNNVKTVREILMEFERLYEYDIPFVRRYLIDNSVIPTSTWDFENNKKIDNKIPDFKTVSFAIAVYCNKEPNPKKDPIIMASFSSKDFNTVVSTKKFDHEKLEYVKDEKELIKRIIEILKEYDIIYTYNGDNFDFPYLKKRAESFGLELKLGKNDEKIKITKGGMNSKSYIPGRVHIDLYPIARRLLNLTKYRLENVTEALFDVKKVDVGHENIPKMWDNLDETLVEYSHQDAYYTQRIGEQFLPLEIMFSRVVNQSLYDINRMSSSQMVEYLLLKNSYKMGVIAPNRPSGKEYQKRIRSSYEGGYVKEPLKGIHEDIVSMDFLSLYPSIIMSHNLSPETIDCTCCSDEENGENEEILGHKFCKKSIGIIPKTLMDLINRRKKVKKVLREKAEKGEFDEEYQILDYEQRLIKVLANSHYGYLAFPMARWYSRDCAEITTHLGRQYIQKTIEEAENFGFKVIYADTDGFYSKWADDKEKLSKYELLEKTREFLKNINNTLPGEMELEFEGYFKRGIFVTKKKYALIDENEKITVKGLEVVRRDWSNVSKNTQKNVLNALLKEGSVENAKKVIQDTIKELKDGKVNNEDLLIHTQLTKRIEDYKTTAPHVEVAKKILKSGNRVNTGDVISYIITSGNKSISERAEILENAKNYDTNYYIENQILPPVIRLMEALGITKDELKDSKKQYTLHHFLK

SEQ ID NO: 26 - protein, 784 aa, Methanococcus maripaludis
MESLIDLDYNSDDLCIYLYLINSIIKEKDFKPYFYVNSTDKEQILEFLKDYEKKHKLDSEISKMIENIETVKKIVFDENYQEKELSKVTVKYPNNVKTVREILMEFERLYEYDIPFVRRYLIDNSVIPTSTWDFENNKKIDNKIPDFKTVSFAIAVYCNKEPNPKKDPIIMASFSSKDFNTVVSTKKFDHEKLEYVKDEKELIKRIIEILKEYDIIYTYNGDNFDFPYLKKRAESFGLELKLGKNDEKIKITKGGMNSKSYIPGRVHIDLYPIARRLLNLTKYRLENVTEALFDVKKVDVGHENIPKMWDNLDETLVEYSHQDAYYTQRIGEQFLPLEIMFSRVVNQSLYDINRMSSSQMVEYLLLKNSYKMGVIAPNRPSGKEYQKRIRSSYEGGYVKEPLKGIHEDIVSMDFLSLYPSIIMSHNLSPETIDCTCCSDEENGENEEILGHKFCKKSIGIIPKTLMDLINRRKKVKKVLREKAEKGEFDEEYMILDYEQRLIKVLANSHYGYLAFPMARWYSRDCAEITTHLGRQYIQKTIEEAENFGFKVIYADTDGFYSKWADDKEKLSKYELLEKTREFLKNINNTLPGEMELEFEGYFKRGIFVTKKKYALIDENEKITVKGLEVVRRDWSNVSKNTQKNVLNALLKEGSVENAKKVIQDTIKELKDGKVNNEDLLIHTQLTKRIEDYKTTAPHVEVAKKILKSGNRVNTGDVISYIITSGNKSISERAEILENAKNYDTNYYIENQILPPVIRLMEALGITKDELKDSKKQYTLHHFLK

SEQ ID NO: 27 - protein, 784 aa, Methanococcus maripaludis
  VARIANT (419)..(419): X=I, V, A
MESLIDLDYNSDDLCIYLYLINSIIKEKDFKPYFYVNSTDKEQILEFLKDYEKKHKLDSEISKMIENIETVKKIVFDENYQEKELSKVTVKYPNNVKTVREILMEFERLYEYDIPFVRRYLIDNSVIPTSTWDFENNKKIDNKIPDFKTVSFAIAVYCNKEPNPKKDPIIMASFSSKDFNTVVSTKKFDHEKLEYVKDEKELIKRIIEILKEYDIIYTYNGDNFDFPYLKKRAESFGLELKLGKNDEKIKITKGGMNSKSYIPGRVHIDLYPIARRLLNLTKYRLENVTEALFDVKKVDVGHENIPKMWDNLDETLVEYSHQDAYYTQRIGEQFLPLEIMFSRVVNQSLYDINRMSSSQMVEYLLLKNSYKMGVIAPNRPSGKEYQKRIRSSYEGGYVKEPLKGIHEDIVSMDFLSAAXSIIMSHNLSPETIDCTCCSDEENGENEEILGHKFCKKSIGIIPKTLMDLINRRKKVKKVLREKAEKGEFDEEYMILDYEQRLIKVLANSHYGYLAFPMARWYSRDCAEITTHLGRQYIQKTIEEAENFGFKVIYADTDGFYSKWADDKEKLSKYELLEKTREFLKNINNTLPGEMELEFEGYFKRGIFVTKKKYALIDENEKITVKGLEVVRRDWSNVSKNTQKNVLNALLKEGSVENAKKVIQDTIKELKDGKVNNEDLLIHTQLTKRIEDYKTTAPHVEVAKKILKSGNRVNTGDVISYIITSGNKSISERAEILENAKNYDTNYYIENQILPPVIRLMEALGITKDELKDSKKQYTLHHFLK

SEQ ID NO: 28 - protein, 784 aa, Methanococcus maripaludis
MESLIDLDYNSDDLCIYLYLINSIIKEKDFKPYFYVNSTDKEQILEFLKDYEKKHKLDSEISKMIENIETVKKIVFDENYQEKELSKVTVKYPNNVKTVREILMEFERLYEYDIPFVRRYLIDNSVIPTSTWDFENNKKIDNKIPDFKTVSFAIAVYCNKEPNPKKDPIIMASFSSKDFNTVVSTKKFDHEKLEYVKDEKELIKRIIEILKEYDIIYTYNGDNFDFPYLKKRAESFGLELKLGKNDEKIKITKGGMNSKSYIPGRVHIDLYPIARRLLNLTKYRLENVTEALFDVKKVDVGHENIPKMWDNLDETLVEYSHQDAYYTQRIGEQFLPLEIMFSRVVNQSLYDINRMSSSQMVEYLLLKNSYKMGVIAPNRPSGKEYQKRIRSSYEGGYVKEPLKGIHEDIVSMDFLSLAPSIIMSHNLSPETIDCTCCSDEENGENEEILGHKFCKKSIGIIPKTLMDLINRRKKVKKVLREKAEKGEFDEEYMILDYEQRLIKVLANSHYGYLAFPMARWYSRDCAEITTHLGRQYIQKTIEEAENFGFKVIYADTDGFYSKWADDKEKLSKYELLEKTREFLKNINNTLPGEMELEFEGYFKRGIFVTKKKYALIDENEKITVKGLEVVRRDWSNVSKNTQKNVLNALLKEGSVENAKKVIQDTIKELKDGKVNNEDLLIHTQLTKRIEDYKTTAPHVEVAKKILKSGNRVNTGDVISYIITSGNKSISERAEILENAKNYDTNYYIENQILPPVIRLMEALGITKDELKDSKKQYTLHHFLK

SEQ ID NO: 29 - protein, 775 aa, Thermococcus sp. 9N-7
MILDTDYITENGKPVIRVFKKENGEFKIEYDRTFEPYFYALLKDDSAIEDVKKVTAKRHGTVVKVKRAEKVQKKFLGRPIEVWKLYFNHPQDVPAIRDRIRAHPAVVDIYEYDIPFAKRYLIDKGLIPAEGDEELTMLAFAIATLYHEGEEFGTGPILMISYADGSEARVITWKKIDLPYVDVVSTEKEMIKRFLRVVREKDPDVLITYNGDNFDFAYLKKRSEELGIKFTLGRDGSEPKIQRMGDRFAVEVKGRIHFDLYPVIRRTINLPTYTLEAVYEAVFGKPKEKVYAEEIAQAWESGEGLERVARYSMEDAKVTYELGREFFPMEAQLSRLIGQSLWDVSRSSTGNLVEWFLLRKAYKRNELAPNKPDERELARRRGGYAGGYVKEPERGLWDNIVYLDFRSAAISIIITHNVSPDTLNREGCKEYDVAPEVGHKFCKDFPGFIPSLLGDLLEERQKIKRKMKATVDPLEKKLLDYRQRVIKILANSFYGYYGYAKARWYCKECAESVSAWGREYLEMVIRELEEKFGFKVLYADTDGLHATIPGADAETVKKKAKEFLKYINPKLPGLLELEYEGFYVRGFFVTKKKYAVIDEEGKITTRGLEIVRRDWSEIAKETQARVLEAILKHGDVEEAVRIVKEVTEKLSKYEVPPEKLVIHEQITRDLRDYKATGPHVAVAKRLAARGVKIRPGTVISYIVLKGSGRIGDRAIPADEFDPTKHRYDAEYYIENQVLPAVERILKAFGYRKEDLRYQKTKQVGLGAWLKVKGKK

SEQ ID NO: 30 - protein, 775 aa, Thermococcus sp. 9N-7
MILDTDYITENGKPVIRVFKKENGEFKIEYDRTFEPYFYALLKDDSAIEDVKKVTAKRHGTVVKVKRAEKVQKKFLGRPIEVWKLYFNHPQDVPAIRDRIRAHPAVVDIYEYDIPFAKRYLIDKGLIPAEGDEELTMLAFAIATLYHEGEEFGTGPILMISYADGSEARVITWKKIDLPYVDVVSTEKEMIKRFLRVVREKDPDVLITYNGDNFDFAYLKKRSEELGIKFTLGRDGSEPKIQRMGDRFAVEVKGRIHFDLYPVIRRTINLPTYTLEAVYEAVFGKPKEKVYAEEIAQAWESGEGLERVARYSMEDAKVTYELGREFFPMEAQLSRLIGQSLWDVSRSSTGNLVEWFLLRKAYKRNELAPNKPDERELARRRGGYAGGYVKEPERGLWDNIVYLDFRSAAISIIITHNVSPDTLNREGCKEYDVAPEVGHKFCKDFPGFIPSLLGDLLEERQKIKRKMKATVDPLEKMLLDYRQRVIKILANSFYGYYGYAKARWYCKECAESVSAWGREYLEMVIRELEEKFGFKVLYADTDGLHATIPGADAETVKKKAKEFLKYINPKLPGLLELEYEGFYVRGFFVTKKKYAVIDEEGKITTRGLEIVRRDWSEIAKETQARVLEAILKHGDVEEAVRIVKEVTEKLSKYEVPPEKLVIHEQITRDLRDYKATGPHVAVAKRLAARGVKIRPGTVISYIVLKGSGRIGDRAIPADEFDPTKHRYDAEYYIENQVLPAVERILKAFGYRKEDLRYQKTKQVGLGAWLKVKGKK

SEQ ID NO: 31 - protein, 775 aa, Thermococcus sp. 9N-7
MILDTDYITENGKPVIRVFKKENGEFKIEYDRTFEPYFYALLKDDSAIEDVKKVTAKRHGTVVKVKRAEKVQKKFLGRPIEVWKLYFNHPQDVPAIRDRIRAHPAVVDIYEYDIPFAKRYLIDKGLIPAEGDEELTMLAFAIATLYHEGEEFGTGPILMISYADGSEARVITWKKIDLPYVDVVSTEKEMIKRFLRVVREKDPDVLITYNGDNFDFAYLKKRSEELGIKFTLGRDGSEPKIQRMGDRFAVEVKGRIHFDLYPVIRRTINLPTYTLEAVYEAVFGKPKEKVYAEEIAQAWESGEGLERVARYSMEDAKVTYELGREFFPMEAQLSRLIGQSLWDVSRSSTGNLVEWFLLRKAYKRNELAPNKPDERELARRRGGYAGGYVKEPERGLWDNIVYLDFRSAAISIIITHNVSPDTLNREGCKEYDVAPEVGHKFCKDFPGFIPSLLGDLLEERQKIKRKMKATVDPLEKKLLDYRQRVIKILANSFYGYYGYAKARWYCKECAESVAAWGREYLEMVIRELEEKFGFKVLYADTDGLHATIPGADAETVKKKAKEFLKYINPKLPGLLELEYEGFYVRGFFVTKKKYAVIDEEGKITTRGLEIVRRDWSEIAKETQARVLEAILKHGDVEEAVRIVKEVTEKLSKYEVPPEKLVIHEQITRDLRDYKATGPHVAVAKRLAARGVKIRPGTVISYIVLKGSGRIGDRAIPADEFDPTKHRYDAEYYIENQVLPAVERILKAFGYRKEDLRYQKTKQVGLGAWLKVKGKK

SEQ ID NO: 32 - protein, 775 aa, Thermococcus sp. 9N-7
MILDTDYITENGKPVIRVFKKENGEFKIEYDRTFEPYFYALLKDDSAIEDVKKVTAKRHGTVVKVKRAEKVQKKFLGRPIEVWKLYFNHPQDVPAIRDRIRAHPAVVDIYEYDIPFAKRYLIDKGLIPAEGDEELTMLAFAIATLYHEGEEFGTGPILMISYADGSEARVITWKKIDLPYVDVVSTEKEMIKRFLRVVREKDPDVLITYNGDNFDFAYLKKRSEELGIKFTLGRDGSEPKIQRMGDRFAVEVKGRIHFDLYPVIRRTINLPTYTLEAVYEAVFGKPKEKVYAEEIAQAWESGEGLERVARYSMEDAKVTYELGREFFPMEAQLSRLIGQSLWDVSRSSTGNLVEWFLLRKAYKRNELAPNKPDERELARRRGGYAGGYVKEPERGLWDNIVYLDFRSAAISIIITHNVSPDTLNREGCKEYDVAPEVGHKFCKDFPGFIPSLLGDLLEERQKIKRKMKATVDPLEKMLLDYRQRVIKILANSFYGYYGYAKARWYCKECAESVAAWGREYLEMVIRELEEKFGFKVLYADTDGLHATIPGADAETVKKKAKEFLKYINPKLPGLLELEYEGFYVRGFFVTKKKYAVIDEEGKITTRGLEIVRRDWSEIAKETQARVLEAILKHGDVEEAVRIVKEVTEKLSKYEVPPEKLVIHEQITRDLRDYKATGPHVAVAKRLAARGVKIRPGTVISYIVLKGSGRIGDRAIPADEFDPTKHRYDAEYYIENQVLPAVERILKAFGYRKEDLRYQKTKQVGLGAWLKVKGKK